European Patent Application EP 4 512 894 A1, published February 26, 2025. Title: Fructanase variants. Applicant: AB Enzymes Oy. The sequence listing filed with the application follows.

SEQUENCE LISTING (23 sequences)

SEQ ID NO: 1 - protein, 1328 aa, Streptococcus sobrinus
EDTTATTASSSSTQLADAGGISEKSADNSATTSTSATDNPTTVADKQTTPESQDASTGDETSKSDVTPESGETDGKAAADTSTAAVSVEANEQTDVDSSKGETSTVKPADVAVTLEKADAAQVAEKGYQTNLTNLKPTNGTWEVRDDGLYSNAIDKGDSWELSDIQADNFVYSTDVKFLKDQGAVGLIFRSTDPNNVQNSYAINIDGGTKKSKFWRWQDGQDQQLIDEKEISPSDDGNYFIRVVALDSWLSFYINGQLIGSTGDYTLQKDDRGQTTVIKDGYLGLLNWNSEVVFQNTYYTPITDDLNPELEDVTVTSDQGSVEKKGQFLANAPINIQYVDNATTSVKLTIKPKNNQADIKITDSTGKEYQLTDSIPLAVGANYLTVTSTVTTEANQASLTYRINVHRRQANDVYYNELFRDQYHYSVKDGWGNDPNGLVYYKGKYHLFYQFYDDNVWGPMHWAHATSTDLIHWEEQPIALYPDTNGTMFSGCIVVDEHNTSGFFKDGEGGLVALVTADGNGQRIKLAYSSDEGQTWTKVDQVAADWSNDPLQSKDFRDPKVFHWNNKWFMVLAGGPLRIYSSDNLRDWSVESTYPDIQTECPDLYPIQTDDGTVKWVLSRGGRYYKVGDFKQVDGKWTFCPDQAYQDSDGIMNFGKDSYAAMTYYVQDFGSEANPTIPKLTELNWMNTWDYCNLVGKTLDQDFNGTYNLNLQLGLTKENDRYVLTQTPIKAYESLRDTAKAINYQDVTVSANNDLLKDVKSDSYEIVSTFRPSASTTKVGFKLRQSQDQVTVVSYDLQTQELSIDRSKSGIIINDKFAEVNKQKVTTNADGSISLHIFVDRASLEVFAKGDTVAGANQIFPAPDSLGASVFTEGGDAKADIAFYPLKSIWTNKVVTDKPFKLVGTGQAETRLNTGQSTSFEAYLAPAQAKQEVNWQLDKPDLVDFSQSGNKVTLTAKKAGSLTLTASSKEDPSLTKVYKINIFENNFKTNLKNLKAISGQWVVDDKELLDSNTSANDAIMSTDIVPYAEYKLEADVKYQKGLVNIFFASPATDPANAYTFQLGDQTSARLYYFQGDTITEEPLTKALNDNLYHHLEIKKTKDSVSLSVDGQEVMSHKFDTVKDYFNKAYIGLGLWDGEVAFQNVYLTPLNQEVKSQGWFTANQAWYYRKADGQLETGLADIDGQTHYFNADGSQVKGDFASPDGGKTWYYLDKDNGQVLTGLQVINGKTYYFNADGSQVKGDFASPDGGKTWYYLDKDNGQALTGGQTIAGKRYTFDETGQQIKGRFVTPDGGITWYYLDKDNGLRVTGRQVINDEVCYFDQDGRQLK

SEQ ID NO: 2 - protein, 1152 aa, synthetic construct
EDTTATTASSSSTQLADAGGISEKSADNSATTSTSATDNPTTVADKQTTPESQDASTGDETSKSDVTPESGETDGKAAADTSTAAVSVEANEQTDVDSSKGETSTVKPADVAVTLEKADAAQVAEKGYQTNLTNLKPTNGTWEVRDDGLYSNAIDKGDSWELSDIQADNFVYSTDVKFLKDQGAVGLIFRSTDPNNVQNSYAINIDGGTKKSKFWRWQDGQDQQLIDEKEISPSDDGNYFIRVVALDSWLSFYINGQLIGSTGDYTLQKDDRGQTTVIKDGYLGLLNWNSEVVFQNTYYTPITDDLNPELEDVTVTSDQGSVEKKGQFLANAPINIQYVDNATTSVKLTIKPKNNQADIKITDSTGKEYQLTDSIPLAVGANYLTVTSTVTTEANQASLTYRINVHRRQANDVYYNELFRDQYHYSVKDGWGNDPNGLVYYKGKYHLFYQFYDDNVWGPMHWAHATSTDLIHWEEQPIALYPDTNGTMFSGCIVVDEHNTSGFFKDGEGGLVALVTADGNGQRIKLAYSSDEGQTWTKVDQVAADWSNDPLQSKDFRDPKVFHWNNKWFMVLAGGPLRIYSSDNLRDWSVESTYPDIQTECPDLYPIQTDDGTVKWVLSRGGRYYKVGDFKQVDGKWTFCPDQAYQDSDGIMNFGKDSYAAMTYYVQDFGSEANPTIPKLTELNWMNTWDYCNLVGKTLDQDFNGAYNLNLQLGLTKENDRYVLTQTPIKAYESLRDTAKAINYQDVTVSANNDLLKDVKSDSYEIVSTFRPSASTTKVGFKLRQSQDQVTVVSYDLQTQELSIDRSKSGIIINDKFAEVNKQKVTTNADGSISLHIFVDRASLEVFAKGDTVAGANQIFPAPDSLGASVFTEGGDAKADIAFYPLKSIWTNKVVTDKPFKLVGTGQAETRLNTGQSTSFEAYLAPAQAKQEVNWQLDKPDLVDFSQSGNKVTLTAKKAGSLTLTASSKEDPSLTKVYKINIFENNFKTNLKNLKAISGQWVVDDKELLDSNTSANDAIMSTDIVPYAEYKLEADVKYQKGLVNIFFASPATDPANAYTFQLGDQTSARLYYFQGDTITEEPLTKALNDNLYHHLEIKKTKDSVSLSVDGQEVMSHKFDTVKDYFNKAYIGLGLWDGEVAFQNVYLTPLNQE

SEQ ID NO: 3 - protein, 1418 aa, Streptococcus parvulus
MEDQHDTSYKKWFMGKIGTHRIAGCLLAALGAFMLQIGIFGVQEAFANPTSTSSPVVEVRQQDTSPDSSLGSTEKSAQTNQTVHVDQDAEANQTSDDVKQTSAEAQDKNQSTDEVKNDKVDVAEKKEEVPALSSAVESENKTEVSAVSAENQSGFKTNLEDTHGDQNGNWEAREDGLYSDARGKGDSFFYSQSKGKNFVYSTDVTFLSKEGAAALVFRSNNDPNNKNSYAVNIDGGSNNVKFWRWQGGRDYQFINEKHIEPTADNTYHLKVVSIGSWTSYYVNDVLVASLGDYTLQRDDKGQNTYISEGYYGLLNWNSQVRFQNTFYKEITEEESPELKDITVTSKTGTVEQKGQFTSPVTIQYVKNNAASIDLNIQPKNSAAKIQVTDAAGHVYSDFKNIPLAVGANYLTVTSTITTDDGQDVSVTYRLNVHRRQADEVYYNELYRDQYHYSVKDGWANDPNGLVYYKGVYHFFYQFHDDTKWGPMHWGHATSTDLVHWKEQPIAFYPDANGAMFSGSIVADPNNTSGLFDNGEGGLVALITADGNGQRIKLAYSKDEGRTWTKVDQVAADWTDDPLQSQDFRDPKVFRWQNKWFMVVAGGPLRIYSSDNLRNWKVESTYPNLHTECPDLYPIKANDGTIKWVLSRGGRFYKVGDFKQVDGKWTFVPDAEFEQADQSMNFGKDSYAAMTYYVQDFGTTENPTLPELVEVNWMNTWDDYCNLVANTVGQKFNGTFNLNLKLGLVKQDGSYRLTQTPIDAYKSLRQEDKAITLKDVDIDEKSDALKGFSGDQYEIVSTFRPGKDTKKVGFNLRVGGNEVTRVVYDLETETLSIDRSKSGIILSNKFAQVDSQSVKRNADGSIDLHIYVDRASVEVFSRGNTVAGANQIFPAPSSLGVSAFAEGGTAKADITLYPLASTWTDKKEATKPLELVQASPVQNNVYVGDTVELKAYVMPSTVPQDVVWSVDNPDLVSVKEEGNKLLVTALKKGTVKITATSKSDPTLSKEFTVSISRNDFKTNVKDLTSVAGKWYVDGESLYDKNVSANDYYMGKQKIPFPEYELDVDIKYQKGLINIFYASENVDPRNAYSVQFGDNDAVRLYRFMGDTIAEGSMNGKRLNDGKFHHVKVIKGKNSVKVLVDGVEYLNHTFDTVDSYYNNAYVGLGLWDGDLEVQNLFVTNPHASKVNKENLQKAVDKANDVDISLYTEETVRAYQEALAQAKQVLANENVEQSAVDAAAQNLNDVFGKLSAKLVYQVTPDEGVKELVFSKPVVNIITETIPFKRQERTNPNLKQGLRRLITAGKNGLRRILVEVSGDDRRVIEDSTVDSAIDEIVEVGTQTASQNGTNNQQTAPNDAVTTNETSAVNQLAQTTTTDTSTKTSDGSLPNTGVVDQVAVSAGLTLLGSGLVAGSRKKKRDKLD

SEQ ID NO: 4 - protein, 1030 aa, synthetic construct
QSGFKTNLEDTHGDQNGNWEAREDGLYSDARGKGDSFFYSQSKGKNFVYSTDVTFLSKEGAAALVFRSNNDPNNKNSYAVNIDGGSNNVKFWRWQGGRDYQFINEKHIEPTADNTYHLKVVSIGSWTSYYVNDVLVASLGDYTLQRDDKGQNTYISEGYYGLLNWNSQVRFQNTFYKEITEEESPELKDITVTSKTGTVEQKGQFTSPVTIQYVKNNAASIDLNIQPKNSAAKIQVTDAAGHVYSDFKNIPLAVGANYLTVTSTITTDDGQDVSVTYRLNVHRRQADEVYYNELYRDQYHYSVKDGWANDPNGLVYYKGVYHFFYQFHDDTKWGPMHWGHATSTDLVHWKEQPIAFYPDANGAMFSGSIVADPNNTSGLFDNGEGGLVALITADGNGQRIKLAYSKDEGRTWTKVDQVAADWTDDPLQSQDFRDPKVFRWQNKWFMVVAGGPLRIYSSDNLRNWKVESTYPNLHTECPDLYPIKANDGTIKWVLSRGGRFYKVGDFKQVDGKWTFVPDAEFEQADQSMNFGKDSYAAMTYYVQDFGTTENPTLPELVEVNWMNTWDDYCNLVANTVGQKFNGAFNLNLKLGLVKQDGSYRLTQTPIDAYKSLRQEDKAITLKDVDIDEKSDALKGFSGDQYEIVSTFRPGKDTKKVGFNLRVGGNEVTRVVYDLETETLSIDRSKSGIILSNKFAQVDSQSVKRNADGSIDLHIYVDRASVEVFSRGNTVAGANQIFPAPSSLGVSAFAEGGTAKADITLYPLASTWTDKKEATKPLELVQASPVQNNVYVGDTVELKAYVMPSTVPQDVVWSVDNPDLVSVKEEGNKLLVTALKKGTVKITATSKSDPTLSKEFTVSISRNDFKTNVKDLTSVAGKWYVDGESLYDKNVSANDYYMGKQKIPFPEYELDVDIKYQKGLINIFYASENVDPRNAYSVQFGDNDAVRLYRFMGDTIAEGSMNGKRLNDGKFHHVKVIKGKNSVKVLVDGVEYLNHTFDTVDSYYNNAYVGLGLWDGDLEVQNLFVTNPHAS

SEQ ID NO: 5 - protein, 1242 aa, Clostridium pasteurianum
ETISTFTREDFINGEFGNTDNGLELLKKDGDNAAITSTYSEKFSYEADVNLEDGPSAALIFGVANKDNPSSGVWYGVNINKTEGYSYAENDKVTGVIRMFKVVPGQDLGINEAVPLTEAQKAKNTFHYKVTVDSNKNIKFYLDGNLVFVKNDPSWTGGNAGLLTFNTKATFSNIKFSDSPVDNDENGFSTNLTNITGLKGTWIKTNEGLFSQGRGDSFAISDTTGSDFIYQTDVTLPSVGAASIVFRSNDNGSDSYVANVDSGAGMGKLFKFQNGSATVFKEFKIPSKSTYNLKVKAIGSHVDYYIDNNLVGSFDDSSFSSGKFGLLNYSASEIYQNLNKTDINAATYPKLTDLKIEGVNLSPSFSENVFNYNANTEYTVDKIKLKLSAVNASSVKVRVLDSKGIEVFNKDLQNNTFNEIAIPVGLNKVYVTAKDNEDNERTYLINLKRALDPTSYYSEEFRPQFHYSPKENWLNDPNGMVYYEGEYHLFYQYYPYGKEWGPMHWGHAVTKDLIHWTELPIALYPDDIGAIFSGSAVVDENNTTGFFTNTSEKKGLVAIYTTDNSGIQQQNVAYSTDKGRTWIKYTGNPVLKTSDDPLNNGAFRDPKVFWDEDAKKWIMVVAGGPLRFFSSSDLKNWKAEAMQPEIETECPDFLRMKVEGTNEYKWVLSGGGRFYMIGDFKEVNGKLTFVPEADKISMNFGRDSYAGQTYNNTPDGRVIMINWMNTWDNYCKAVSAITEPFNGNFNLQLELKLKKNLQGQIKLIQEPIKEYDSLRLAPTVIENATVGSTGNVLQGITGKQTEIVAEFTPGAATTDVGFKLRVGNNQETVVNYNIATKKVSIDRSKSGKIPTENGNRYYESDLFKAVETGDMSMTSDGKIKLKIYLDWASIEVFGNEGEVTGASLIFPDSSSTAMETYSKGEDSKANITLYPMDSIWKSSSSSLSVKAVDSANNNKLLKDAEFKLYDANGNAIGTDNIKTDSKGQVSINNLAPAEYVLKQVKAPKAYNLEESFSQKIDLTKGNQSVDVNFVKAANPEKEAYKVVFKDYDGTVLSEQEVKSGKSAKAPKKPVREGYDFTGWDKSFHKVTEDLVVTAVYKVKTYTVIFKDYKGKTIGKAQTVEYGSAAKAPEAPAREGYTFTGWNKDFSNVKKNLEVKAEYKINSYTVVFKDYNGEIIGKPQTVEYGKSAKAPKAPRRPGYVFTGWDKNFNNVKGDLEVKATYHKVNAWSGVFYRNIWTWIISIF

SEQ ID NO: 6 - protein, 1242 aa, synthetic construct
ETISTFTREDFINGEFGNTDNGLELLKKDGDNAAITSTYSEKFSYEADVNLEDGPSAALIFGVANKDNPSSGVWYGVNINKTEGYSYAENDKVTGVIRMFKVVPGQDLGINEAVPLTEAQKAKNTFHYKVTVDSNKNIKFYLDGNLVFVKNDPSWTGGNAGLLTFNTKATFSNIKFSDSPVDNDENGFSTNLTNITGLKGTWIKTNEGLFSQGRGDSFAISDTTGSDFIYQTDVTLPSVGAASIVFRSNDNGSDSYVANVDSGAGMGKLFKFQNGSATVFKEFKIPSKSTYNLKVKAIGSHVDYYIDNNLVGSFDDSSFSSGKFGLLNYSASEIYQNLNKTDINAATYPKLTDLKIEGVNLSPSFSENVFNYNANTEYTVDKIKLKLSAVNASSVKVRVLDSKGIEVFNKDLQNNTFNEIAIPVGLNKVYVTAKDNEDNERTYLINLKRALDPTSYYSEEFRPQFHYSPKENWLNDPNGMVYYEGEYHLFYQYYPYGKEWGPMHWGHAVTKDLIHWTELPIALYPDDIGAIFSGSAVVDENNTTGFFTNTSEKKGLVAIYTTDNSGIQQQNVAYSTDKGRTWIKYTGNPVLKTSDDPLNNGAFRDPKVFWDEDAKKWIMVVAGGPLRFFSSSDLKNWKAEAMQPEIETECPDFLRMKVEGTNEYKWVLSGGGRFYMIGDFKEVNGKLTFVPEADKISMNFGRDSYAGQTYNNAPDGRVIMINWMNTWDNYCKAVSAITEPFNGNFNLQLELKLKKNLQGQIKLIQEPIKEYDSLRLAPTVIENATVGSTGNVLQGITGKQTEIVAEFTPGAATTDVGFKLRVGNNQETVVNYNIATKKVSIDRSKSGKIPTENGNRYYESDLFKAVETGDMSMTSDGKIKLKIYLDWASIEVFGNEGEVTGASLIFPDSSSTAMETYSKGEDSKANITLYPMDSIWKSSSSSLSVKAVDSANNNKLLKDAEFKLYDANGNAIGTDNIKTDSKGQVSINNLAPAEYVLKQVKAPKAYNLEESFSQKIDLTKGNQSVDVNFVKAANPEKEAYKVVFKDYDGTVLSEQEVKSGKSAKAPKKPVREGYDFTGWDKSFHKVTEDLVVTAVYKVKTYTVIFKDYKGKTIGKAQTVEYGSAAKAPEAPAREGYTFTGWNKDFSNVKKNLEVKAEYKINSYTVVFKDYNGEIIGKPQTVEYGKSAKAPKAPRRPGYVFTGWDKNFNNVKGDLEVKATYHKVNAWSGVFYRNIWTWIISIF

SEQ ID NO: 7 - protein, 483 aa, synthetic construct
SYYSEEFRPQFHYSPKENWLNDPNGMVYYEGEYHLFYQYYPYGKEWGPMHWGHAVTKDLIHWTELPIALYPDDIGAIFSGSAVVDENNTTGFFTNTSEKKGLVAIYTTDNSGIQQQNVAYSTDKGRTWIKYTGNPVLKTSDDPLNNGAFRDPKVFWDEDAKKWIMVVAGGPLRFFSSSDLKNWKAEAMQPEIETECPDFLRMKVEGTNEYKWVLSGGGRFYMIGDFKEVNGKLTFVPEADKISMNFGRDSYAGQTYNNAPDGRVIMINWMNTWDNYCKAVSAITEPFNGNFNLQLELKLKKNLQGQIKLIQEPIKEYDSLRLAPTVIENATVGSTGNVLQGITGKQTEIVAEFTPGAATTDVGFKLRVGNNQETVVNYNIATKKVSIDRSKSGKIPTENGNRYYESDLFKAVETGDMSMTSDGKIKLKIYLDWASIEVFGNEGEVTGASLIFPDSSSTAMETYSKGEDSKANITLYPMDSIWK

SEQ ID NO: 8 - protein, 1049 aa, Lachnospiraceae bacterium
YFFNKPAPPQENPVLEEYVDPALTEGVFNTNLTGITFAGGKWEGTDEGLHSTALGAGDCFLYSNTSAKNFIYSVDVKFLKDEGAASLVFRGDERGSHYNCYAVNLDAGSKLIKFWRWFKGDAGQLSSELKVEERPDKCYNLKVVVIDSWVSYFVNDVLMASSGDYILSGDARGQYTVPEEGYLGLLNWNGDMIFQNAYYTPIEDDAKPYLKSMTVRASGGSAEASSQFSFDEPITLQYVDNDTETVDIAAEAFSKDAVITVAGPDGREYEGGKGIPVEVGKNIITVTSTTKADDKDVTLTYRVNVHRRQPEAVYYNEPYRDQYHYSVKDGWGNDPNGLVYYKGTYHLFYQFYDDIAWGPMHWGHAVSKDLITWEEKPIAFYPDTNGAMFSGCIVVDDQNTSGLFKSPEGGLVALITCDGSGQRIKLAYSEDEGETWTKVKQIAADWTDDPLHDGAFRDPKVFRWEGKWFMVIAGGPLRIYSSDNLIDWTCETTYADLHTECPDLYPIQADDGRIKWVLDRGGRAYKVGDFTSESGAWAFVPDQAYADRDAVMNFGKDSYAAMTYYIQDFGTAAEPTLPEIIEINWMNTWDDYCNRVAAAVGQNFNGTYNLFLKEGLVKDGDSYLLTQTPIEAYDSLRGEAIEAKGVSITPESNLFADFRGDTYEIQAVFHPGGNTRKVGFDLRKNGDEKTSVIYDLEAGQIYIDRSRSGIIISRRFADVDRQDVSTDEDGSVTMHIYVDRASVEVFTKNYTVTGANQIFPSADALGLSAVSEGDTSTADITVYPLKSIWTPASSDVPVAMTAPSSGSVVYVGGELTLNTTLIPMTGSQDVGWSVSDESVVSISSEGSRAVVSGLKTGKATVTATAAANEALTKNFEITVLENNFDTNLGEFEAVVGDWIVDDKILTVSNQSSNDFYMAKTPVDQNEYTIDTRIRFTKGFVNIFFAANSMDPFDRQAYAVQVSQGSSSVRIFRFAGDTIFESSMGKAISDDEWHDISIKKTTDSVSVSVDGQEAVTASVADPEDYFNGNPYVGIGIWDGAMEVDGFKIQY

SEQ ID NO: 9 - protein, 1049 aa, synthetic construct
YFFNKPAPPQENPVLEEYVDPALTEGVFNTNLTGITFAGGKWEGTDEGLHSTALGAGDCFLYSNTSAKNFIYSVDVKFLKDEGAASLVFRGDERGSHYNCYAVNLDAGSKLIKFWRWFKGDAGQLSSELKVEERPDKCYNLKVVVIDSWVSYFVNDVLMASSGDYILSGDARGQYTVPEEGYLGLLNWNGDMIFQNAYYTPIEDDAKPYLKSMTVRASGGSAEASSQFSFDEPITLQYVDNDTETVDIAAEAFSKDAVITVAGPDGREYEGGKGIPVEVGKNIITVTSTTKADDKDVTLTYRVNVHRRQPEAVYYNEPYRDQYHYSVKDGWGNDPNGLVYYKGTYHLFYQFYDDIAWGPMHWGHAVSKDLITWEEKPIAFYPDTNGAMFSGCIVVDDQNTSGLFKSPEGGLVALITCDGSGQRIKLAYSEDEGETWTKVKQIAADWTDDPLHDGAFRDPKVFRWEGKWFMVIAGGPLRIYSSDNLIDWTCETTYADLHTECPDLYPIQADDGRIKWVLDRGGRAYKVGDFTSESGAWAFVPDQAYADRDAVMNFGKDSYAAMTYYIQDFGTAAEPTLPEIIEINWMNTWDDYCNRVAAAVGQNFNGAYNLFLKEGLVKDGDSYLLTQTPIEAYDSLRGEAIEAKGVSITPESNLFADFRGDTYEIQAVFHPGGNTRKVGFDLRKNGDEKTSVIYDLEAGQIYIDRSRSGIIISRRFADVDRQDVSTDEDGSVTMHIYVDRASVEVFTKNYTVTGANQIFPSADALGLSAVSEGDTSTADITVYPLKSIWTPASSDVPVAMTAPSSGSVVYVGGELTLNTTLIPMTGSQDVGWSVSDESVVSISSEGSRAVVSGLKTGKATVTATAAANEALTKNFEITVLENNFDTNLGEFEAVVGDWIVDDKILTVSNQSSNDFYMAKTPVDQNEYTIDTRIRFTKGFVNIFFAANSMDPFDRQAYAVQVSQGSSSVRIFRFAGDTIFESSMGKAISDDEWHDISIKKTTDSVSVSVDGQEAVTASVADPEDYFNGNPYVGIGIWDGAMEVDGFKIQY

SEQ ID NO: 10 - protein, 1471 aa, Oscillibacter sp.
AETDSTEAVAVADTAEEAAGVVSEAAAVEAEPDVTEADTVDTVAVPDTAAVEVEADTGDAEAVADASEVEAEADTVDAVAVPDTAAVEAEPDAESVAVLADAAAAEEDAVATLYDVSTGLTDFSSFNHPDLISIDTAAHTVTMDYVEGDHFVVYNGLDHKLNSFVWEADVDIQPGLQIQSAALIFGFPSPAAANSNWYGANLDSTRLGGDNAFRLFGPNIDTNSGGSVEGIDITRTLHLKVDIHATGAFEYSFGNAGATLKVISGQISGWRNGGYVGLLTWNSGATFSNITLEEREEQIEVQPFGTVTTASGFQYHNNIANANLSDLRTQGGTWEARADGLYSNAVGIGDAFLYSQTTGSNFVYSTDVTFLGENAQGAAALILRNADANGHDECYAANIDASSRRCKLWRWQEGMDNQLFGEVQFTGSATNNTYTLTVVAIDTWLSFYVNGELIGSTGDYYKLGGADWGQDTYISSGTFGLLNWNGEMVFQNTTYTPIDGTFNPLLSDITVTSSGTVEQKGQFISTEPITIQYVKNDAATVNIAATSVSSNATVRVYGPDGTEYPDGRNIPVAVGANYIAVQSSVTNADGVTATVTYRVNVHRRQADALYYNEPYRGQYHYSVKDGWANDPNGLVYFNGTYHFFYQFYDDIEWGPMHWAHVTSPDLIHWTEQPIAFYPDANGSMFSGCIVADVNNTSGLFTGNGGGLVALITTNGNGQRIKVAYSTDEGRTWTKVNNIAADWSRDPLYNRDFRDPKVFRWENKWFMVLAGGPLRIYSSDNLLEWQCESTYANLHTECPDLYPLRADDGVIKWVLSRGGRTYKVGDLRQVDGKWTFVPDAAYANEPDNGIMNFGRDSYAAMTYYVQDFGTAANPTLPAIIEINWMNTWDDYCRDVARRVGQVFNGTFNLNLQLGLKNENGKYVLTQTPIQAYETLRGTPAVSLTGAAVTANNTLLSGFSGDCYEIVSKFYPGTATSVGFDLRVGNGEKTAVRYNVTEGRLSIDRSQSGTMISNIFGQVNSQAVARNADGSVDLRVFVDRSSVEVFTKDYTVAGANQIFPAMSSLGAAVVAEGGDATADITIYPMGGTWTERIDSNTPIEITSNNSDTIRLNVGDTLNLRATLLPVSAPQNINWTVSDSSILSVTGSASGNDFSASVLKAGDVTVTATAAANSALTKTFAVHVTANNFDTNIPSFTVNGGEWTIDDQTLSVSNQAANQFYMSSAAVSLREFTLETNIRFTRGAINIFFAAGGVNPFDPQAYAVQFNDSSSFRLFRFGGDDITAPTDMGQQVNDGQFHNVKIRKTANSVTVSVDNVEKLNYTFDSVENFFNDGAFVGIGLWDGALDVQTFRVTENATPGDGGDTPSTPGGDSGNTPSTPSTPGKKSGCYVATSVYGSYDCPEVWTLRRFRDNVLAETWYGRLFIRAYYAVSPTAVRLFGDADWFQSFFRDRLDNLVTELQADGFESTPYDDISW

SEQ ID NO: 11 - protein, 1350 aa, synthetic construct
AETDSTEAVAVADTAEEAAGVVSEAAAVEAEPDVTEADTVDTVAVPDTAAVEVEADTGDAEAVADASEVEAEADTVDAVAVPDTAAVEAEPDAESVAVLADAAAAEEDAVATLYDVSTGLTDFSSFNHPDLISIDTAAHTVTMDYVEGDHFVVYNGLDHKLNSFVWEADVDIQPGLQIQSAALIFGFPSPAAANSNWYGANLDSTRLGGDNAFRLFGPNIDTNSGGSVEGIDITRTLHLKVDIHATGAFEYSFGNAGATLKVISGQISGWRNGGYVGLLTWNSGATFSNITLEEREEQIEVQPFGTVTTASGFQYHNNIANANLSDLRTQGGTWEARADGLYSNAVGIGDAFLYSQTTGSNFVYSTDVTFLGENAQGAAALILRNADANGHDECYAANIDASSRRCKLWRWQEGMDNQLFGEVQFTGSATNNTYTLTVVAIDTWLSFYVNGELIGSTGDYYKLGGADWGQDTYISSGTFGLLNWNGEMVFQNTTYTPIDGTFNPLLSDITVTSSGTVEQKGQFISTEPITIQYVKNDAATVNIAATSVSSNATVRVYGPDGTEYPDGRNIPVAVGANYIAVQSSVTNADGVTATVTYRVNVHRRQADALYYNEPYRGQYHYSVKDGWANDPNGLVYFNGTYHFFYQFYDDIEWGPMHWAHVTSPDLIHWTEQPIAFYPDANGSMFSGCIVADVNNTSGLFTGNGGGLVALITTNGNGQRIKVAYSTDEGRTWTKVNNIAADWSRDPLYNRDFRDPKVFRWENKWFMVLAGGPLRIYSSDNLLEWQCESTYANLHTECPDLYPLRADDGVIKWVLSRGGRTYKVGDLRQVDGKWTFVPDAAYANEPDNGIMNFGRDSYAAMTYYVQDFGTAANPTLPAIIEINWMNTWDDYCRDVARRVGQVFNGAFNLNLQLGLKNENGKYVLTQTPIQAYETLRGTPAVSLTGAAVTANNTLLSGFSGDCYEIVSKFYPGTATSVGFDLRVGNGEKTAVRYNVTEGRLSIDRSQSGTMISNIFGQVNSQAVARNADGSVDLRVFVDRSSVEVFTKDYTVAGANQIFPAMSSLGAAVVAEGGDATADITIYPMGGTWTERIDSNTPIEITSNNSDTIRLNVGDTLNLRATLLPVSAPQNINWTVSDSSILSVTGSASGNDFSASVLKAGDVTVTATAAANSALTKTFAVHVTANNFDTNIPSFTVNGGEWTIDDQTLSVSNQAANQFYMSSAAVSLREFTLETNIRFTRGAINIFFAAGGVNPFDPQAYAVQFNDSSSFRLFRFGGDDITAPTDMGQQVNDGQFHNVKIRKTANSVTVSVDNVEKLNYTFDSVENFFNDGAFVGIGLWDGALDVQTFRVT

SEQ ID NO: 12 - protein, 973 aa, Ligilactobacillus salivarius
DTVNNNQPQTTMQQNSTTNQNIEYTTEKNNLNSMGSTNNKVAVTDQTTKTPKVETSNVETSNVESNIEENQISNSQVKSSSNQVQDITDVKVDNPETGTISKNEDGSLTANSVDKGDSYAFSDETGNDFVYTADVHFNQKQGAASLVFRANKSTDPIDGYIANIEAATHIAKMWRMVNGTGYELLAPTSFKADENGNYTLKVIAYGKNIEYYINDILVGSAGDYVVQKDDRGQPAYKRQGYFGLLTWNGDVTYKNIRYQNLTDKFNPLLKDITVTSNSGNVEDKGQFFSDGTNYIQYVDNKTKTVDFKVVANNPNAKVVAYDLEGNEYTDLKNIPVSVGANYITIVSEIPASDGTTIKATYHVNVHRRQKADVYYKEKYRDQYHYSVKDGWGNDPNGLIYYNGLYHFFYQFYDDVAWGPMHWGHATSKDLIHWNEEPIAFYPDANGAAFSGSIVADTGNTSGLFSGKNGGLVAFITADGGGQRIKLAYSSDEGKTWTKLDDPVLDYSTDDPLKNGAFRDPKVFRWNNKWFMVVAGGPLRIYSSDNLRQWKVETVYSNIDTECPDLYPIQTDDGIKWVLSRGGRYYKVGDFKQVDGSWSFIPDKAYENKDGIMNFGKDSYAAMTYYIQDFGTETKPTLPELVEVNWMNNWDYCRDVATTVGQKFNGTYNLNLKLGLIKEGNKYVLTQTPIDAYKNLRDTEHAMIFKDVDLSSNNNLLKDFKGDTYEIVAHFKPSETTTKVGFKVRVGDGQSTDIIYDLETDTLSIDRSKSGIQINNLFSLVNSQEVTTNEDGSIDLHLYIDKASVEVFSKGNTVAGTNQIFPDEDSLGASVLVEGGNVKADIAIYPLKSIWFEEENTTNGDDSADKSNTVGKETSKENTNSVDNSSQGEVNNNLTVTGKDNITNLSKDKNTTTLSTAKEKAIESNKRANNLKEANTLPQMGETNSKAEVSTGIVALALSFFGLIFSSVRKRKQK

SEQ ID NO: 13 - protein, 973 aa, synthetic construct
DTVNNNQPQTTMQQNSTTNQNIEYTTEKNNLNSMGSTNNKVAVTDQTTKTPKVETSNVETSNVESNIEENQISNSQVKSSSNQVQDITDVKVDNPETGTISKNEDGSLTANSVDKGDSYAFSDETGNDFVYTADVHFNQKQGAASLVFRANKSTDPIDGYIANIEAATHIAKMWRMVNGTGYELLAPTSFKADENGNYTLKVIAYGKNIEYYINDILVGSAGDYVVQKDDRGQPAYKRQGYFGLLTWNGDVTYKNIRYQNLTDKFNPLLKDITVTSNSGNVEDKGQFFSDGTNYIQYVDNKTKTVDFKVVANNPNAKVVAYDLEGNEYTDLKNIPVSVGANYITIVSEIPASDGTTIKATYHVNVHRRQKADVYYKEKYRDQYHYSVKDGWGNDPNGLIYYNGLYHFFYQFYDDVAWGPMHWGHATSKDLIHWNEEPIAFYPDANGAAFSGSIVADTGNTSGLFSGKNGGLVAFITADGGGQRIKLAYSSDEGKTWTKLDDPVLDYSTDDPLKNGAFRDPKVFRWNNKWFMVVAGGPLRIYSSDNLRQWKVETVYSNIDTECPDLYPIQTDDGIKWVLSRGGRYYKVGDFKQVDGSWSFIPDKAYENKDGIMNFGKDSYAAMTYYIQDFGTETKPTLPELVEVNWMNNWDYCRDVATTVGQKFNGAYNLNLKLGLIKEGNKYVLTQTPIDAYKNLRDTEHAMIFKDVDLSSNNNLLKDFKGDTYEIVAHFKPSETTTKVGFKVRVGDGQSTDIIYDLETDTLSIDRSKSGIQINNLFSLVNSQEVTTNEDGSIDLHLYIDKASVEVFSKGNTVAGTNQIFPDEDSLGASVLVEGGNVKADIAIYPLKSIWFEEENTTNGDDSADKSNTVGKETSKENTNSVDNSSQGEVNNNLTVTGKDNITNLSKDKNTTTLSTAKEKAIESNKRANNLKEANTLPQMGETNSKAEVSTGIVALALSFFGLIFSSVRKRKQK

SEQ ID NO: 14 - protein, 855 aa, Ligilactobacillus salivarius
DTVNNNQPQTTMQQNSTTNQNIEYTTEKNNLNSMGSTNNKVAVTDQTTKTPKVETSNVETSNVESNIEENQISNSQVKSSSNQVQDITDVKVDNPETGTISKNEDGSLTANSVDKGDSYAFSDETGNDFVYTADVHFNQKQGAASLVFRANKSTDPIDGYIANIEAATHIAKMWRMVNGTGYELLAPTSFKADENGNYTLKVIAYGKNIEYYINDILVGSAGDYVVQKDDRGQPAYKRQGYFGLLTWNGDVTYKNIRYQNLTDKFNPLLKDITVTSNSGNVEDKGQFFSDGTNYIQYVDNKTKTVDFKVVANNPNAKVVAYDLEGNEYTDLKNIPVSVGANYITIVSEIPASDGTTIKATYHVNVHRRQKADVYYKEKYRDQYHYSVKDGWGNDPNGLIYYNGLYHFFYQFYDDVAWGPMHWGHATSKDLIHWNEEPIAFYPDANGAAFSGSIVADTGNTSGLFSGKNGGLVAFITADGGGQRIKLAYSSDEGKTWTKLDDPVLDYSTDDPLKNGAFRDPKVFRWNNKWFMVVAGGPLRIYSSDNLRQWKVETVYSNIDTECPDLYPIQTDDGIKWVLSRGGRYYKVGDFKQVDGSWSFIPDKAYENKDGIMNFGKDSYAAMTYYIQDFGTETKPTLPELVEVNWMNNWDYCRDVATTVGQKFNGTYNLNLKLGLIKEGNKYVLTQTPIDAYKNLRDTEHAMIFKDVDLSSNNNLLKDFKGDTYEIVAHFKPSETTTKVGFKVRVGDGQSTDIIYDLETDTLSIDRSKSGIQINNLFSLVNSQEVTTNEDGSIDLHLYIDKASVEVFSKGNTVAGTNQIFPDEDSLGASVLVEGGNVKADIAIYPLKSIWFEEEN

SEQ ID NO: 15 - protein, 855 aa, synthetic construct
DTVNNNQPQTTMQQNSTTNQNIEYTTEKNNLNSMGSTNNKVAVTDQTTKTPKVETSNVETSNVESNIEENQISNSQVKSSSNQVQDITDVKVDNPETGTISKNEDGSLTANSVDKGDSYAFSDETGNDFVYTADVHFNQKQGAASLVFRANKSTDPIDGYIANIEAATHIAKMWRMVNGTGYELLAPTSFKADENGNYTLKVIAYGKNIEYYINDILVGSAGDYVVQKDDRGQPAYKRQGYFGLLTWNGDVTYKNIRYQNLTDKFNPLLKDITVTSNSGNVEDKGQFFSDGTNYIQYVDNKTKTVDFKVVANNPNAKVVAYDLEGNEYTDLKNIPVSVGANYITIVSEIPASDGTTIKATYHVNVHRRQKADVYYKEKYRDQYHYSVKDGWGNDPNGLIYYNGLYHFFYQFYDDVAWGPMHWGHATSKDLIHWNEEPIAFYPDANGAAFSGSIVADTGNTSGLFSGKNGGLVAFITADGGGQRIKLAYSSDEGKTWTKLDDPVLDYSTDDPLKNGAFRDPKVFRWNNKWFMVVAGGPLRIYSSDNLRQWKVETVYSNIDTECPDLYPIQTDDGIKWVLSRGGRYYKVGDFKQVDGSWSFIPDKAYENKDGIMNFGKDSYAAMTYYIQDFGTETKPTLPELVEVNWMNNWDYCRDVATTVGQKFNGAYNLNLKLGLIKEGNKYVLTQTPIDAYKNLRDTEHAMIFKDVDLSSNNNLLKDFKGDTYEIVAHFKPSETTTKVGFKVRVGDGQSTDIIYDLETDTLSIDRSKSGIQINNLFSLVNSQEVTTNEDGSIDLHLYIDKASVEVFSKGNTVAGTNQIFPDEDSLGASVLVEGGNVKADIAIYPLKSIWFEEEN

SEQ ID NO: 16 - protein, 827 aa, Ligilactobacillus equi
MEAASHIAKFWRMVNGQGYELLAPKSYKPTEDGHYNLKVVAYGKNIEYYINDELIGSAGDYVVQKDDKGQPAYKRSGNFGLLTWNGDVTYSNVRYQELTPDFNPFLKDITVVSNEGQAEVKGQFFTDETNYIQYVDNATKTVNLEVLANVPNVQVVAYDQEGNAYTDLKNIPVSVGANYITVVSTVLGADGTPIQASYHVNVHRRQKAEIYYHEPYRDQFHYSVKDGWSNDPNGLVYYNGTYHFFYQFYDDTSWGPMHWGHATSTDLIHWKEEPIALYPDANRAMFSGSIVADVNNTTGLFDQGKGGLVALVTADGGGQRIELAYSKDEGKTWNKLADPVLDYANDDPLHNAAFRDPKVFRWNNQWFMVVAGGPLRIYSSSDLQNWKSESVYSGIETECPDLYPIQTDNGVKWVLSRGGRYYKVGDFKQVDGNWYFLPDKVYEKTDGIMNFGKDSYAAMTYFVQDFGTEANPTLPEIIESNWMNNWDYCNDVAATVGQKFNGTYNLNLKLGLTKEGDKYVLTQTPITAYQDLRDVEHAMTFKNVTVGEDNDLLKDFQGDTYEIVAHFVPAVGTKKLGFNVLTSATQGTSIVYDLEEETMSIDRSKSGKQINAKFTEPNIQNKVTKNADGSVDLHIYVDKASVEVFTKGDTVLGANQIFPDADSLGASLMVEGDPVVADIAIYPLKSIWFADKPVVTPKDDASSSAINDTVNAGEGNVTNVDANISDVNTAANGKNNTVAISNAGDITSEIKVGNNTIILPNSKTKVTLQETEGQSSSVKVQTSKVSVAKQLPQTGEEKTSVWMGVMAALLGALSFLFPAMKRRKGNN

SEQ ID NO: 17 - protein, 689 aa, synthetic construct
MEAASHIAKFWRMVNGQGYELLAPKSYKPTEDGHYNLKVVAYGKNIEYYINDELIGSAGDYVVQKDDKGQPAYKRSGNFGLLTWNGDVTYSNVRYQELTPDFNPFLKDITVVSNEGQAEVKGQFFTDETNYIQYVDNATKTVNLEVLANVPNVQVVAYDQEGNAYTDLKNIPVSVGANYITVVSTVLGADGTPIQASYHVNVHRRQKAEIYYHEPYRDQFHYSVKDGWSNDPNGLVYYNGTYHFFYQFYDDTSWGPMHWGHATSTDLIHWKEEPIALYPDANRAMFSGSIVADVNNTTGLFDQGKGGLVALVTADGGGQRIELAYSKDEGKTWNKLADPVLDYANDDPLHNAAFRDPKVFRWNNQWFMVVAGGPLRIYSSSDLQNWKSESVYSGIETECPDLYPIQTDNGVKWVLSRGGRYYKVGDFKQVDGNWYFLPDKVYEKTDGIMNFGKDSYAAMTYFVQDFGTEANPTLPEIIESNWMNNWDYCNDVAATVGQKFNGAYNLNLKLGLTKEGDKYVLTQTPITAYQDLRDVEHAMTFKNVTVGEDNDLLKDFQGDTYEIVAHFVPAVGTKKLGFNVLTSATQGTSIVYDLEEETMSIDRSKSGKQINAKFTEPNIQNKVTKNADGSVDLHIYVDKASVEVFTKGDTVLGANQIFPDADSLGASLMVEGDPVVADIAIYPLKSIWF

SEQ ID NO: 18 - protein, 1270 aa, Ligilactobacillus equi
MKNVKSTVIYSYSVTTLLAMSAFGISVNHIHADNVTNNTSTAPVTQVSNQTTIQENTNKTAEVPSSESSQATSNGKSQDTSSTPETSAVNTTKQGENNQNIAQNQAEKVQALTDFTYSNNGKWSQQNDGIHSDATGQGDSFAYTDVKGDNFMYSADVTFQKNEGAAALTFRGNNNVDNKDGYAVNVDGGNHKAKFWRWNNNKDYQLIDEKDVTPTDNNTYNLKVIANGHWMEYFVNDTLIASTGDYTLQKDDKGQPTITPEGYFGLLNWNGDVVFKNIKYVTLDNKFSPLLSNISVTSAKGKVEEKGQFASEQPIYIQYVDNDADTVNLQAITKSDKAKVVAYDASGKEYTDLKNIPVHVGANYLTVISEITASDGTKVQAVYRVNVHRRQAQEIYYNELYRDQYHFSVKDGWGNDPNGLVYFNNKYHMFYQFYDDTIWGPMHWAHATSTDLIHWKNEPVAFYPDANGAMFSGSIVVDEGNTSGLFDNAQGGLVAIITADGNGQRIEVAYSKDEGKTWNKLPMIVADWQNDPLQSPDFRDPKVFRWDNKWFMVLAGGPLRIFSSTNLINWQVESEYPDINTECPDLYPVKAVDGQIKWVLSRGGRFYKVGDFHQINGKWTYTPDADYKDQDGIMNFGKDSYAAMTYYQHSFGTQANPTLPDIIENNWMNTWDYCNLVGNTVGQEFNGTYNLNLKLGLVKDGNKYLLTQTPVDAYNSLRDTNKAIVYKNIDVTPNNDLFKDFKGDTYEIVSTFKPSKETTKVGFNVRVGKGQATKVVYDLTSNKIYIDRSQSGVQINNKFTEINEQPVTRNADGSVTLHLYVDRASVEVFTKDDTVTGANQIFPSPQSLGLGVISEGGNSKADIALYPLKSIWTDKEKVTQPLQVVQVSPKNLRLNVGDKTTLTAYVMPGNVQQDLIWKVSDPSLADVTEDGAANSLILDTKNAGHLVVTVASKQDPTLTKDYNIDILANNFKTNVKDLKPLSGNWYVDDVNLHDENVSSNDYIMSSDKIPYPEYDMNVDVKYQKGLANIFFASANQDPNGAYSLQLGGDATLRLYRFYGDTITQTALPYALNDGKVHHVSIHKTKNAVKVSIDGNNVMDYTFDEADPGYNDAYVGLGLWDGSVDFQNFFVNDANKVTEQHESNKDTPTAPSKTNQTPENDSEVTPSKTTTESSTVKDSSDTTKEVSNIPDSKTSVTTPVKTIKLRSQSGNKISIQLPSTTKESKNNKYSQAKKNELPQLSDTQKPGILLGLIMAFSSSVLLFWDKLRRRN

SEQ ID NO: 19 - protein, 873 aa, synthetic construct
MKNVKSTVIYSYSVTTLLAMSAFGISVNHIHADNVTNNTSTAPVTQVSNQTTIQENTNKTAEVPSSESSQATSNGKSQDTSSTPETSAVNTTKQGENNQNIAQNQAEKVQALTDFTYSNNGKWSQQNDGIHSDATGQGDSFAYTDVKGDNFMYSADVTFQKNEGAAALTFRGNNNVDNKDGYAVNVDGGNHKAKFWRWNNNKDYQLIDEKDVTPTDNNTYNLKVIANGHWMEYFVNDTLIASTGDYTLQKDDKGQPTITPEGYFGLLNWNGDVVFKNIKYVTLDNKFSPLLSNISVTSAKGKVEEKGQFASEQPIYIQYVDNDADTVNLQAITKSDKAKVVAYDASGKEYTDLKNIPVHVGANYLTVISEITASDGTKVQAVYRVNVHRRQAQEIYYNELYRDQYHFSVKDGWGNDPNGLVYFNNKYHMFYQFYDDTIWGPMHWAHATSTDLIHWKNEPVAFYPDANGAMFSGSIVVDEGNTSGLFDNAQGGLVAIITADGNGQRIEVAYSKDEGKTWNKLPMIVADWQNDPLQSPDFRDPKVFRWDNKWFMVLAGGPLRIFSSTNLINWQVESEYPDINTECPDLYPVKAVDGQIKWVLSRGGRFYKVGDFHQINGKWTYTPDADYKDQDGIMNFGKDSYAAMTYYQHSFGTQANPTLPDIIENNWMNTWDYCNLVGNTVGQEFNGAYNLNLKLGLVKDGNKYLLTQTPVDAYNSLRDTNKAIVYKNIDVTPNNDLFKDFKGDTYEIVSTFKPSKETTKVGFNVRVGKGQATKVVYDLTSNKIYIDRSQSGVQINNKFTEINEQPVTRNADGSVTLHLYVDRASVEVFTKDDTVTGANQIFPSPQSLGLGVISEGGNSKADIALYPLKSIWT

SEQ ID NO: 20 - protein, 9 aa, unidentified
FNGTYNLFL

SEQ ID NO: 21 - protein, 9 aa, unidentified
FNGTFNLFL

SEQ ID NO: 22 - protein, 9 aa, unidentified
FNGTYNLNL

SEQ ID NO: 23 - protein, 9 aa, unidentified
FNGTFNLNL